European Patent Specification EP 3 990 662 B1, published March 26, 2025. Title: Method for determining the presence or absence of minimal residual disease (MRD) in a subject who has been treated for a disease. Applicant: Fundación para la Investigación Biomédica del Hospital Universitario 12 de Octubre Fundación del Sector Público Estatal Centro Nacional de Investigaciones Oncológicas Carlos III (CNIO). The sequence listing filed with the application follows.

SEQUENCE LISTING (130 sequences)

SEQ ID NO: 1 - DNA, 25 bp, Artificial Sequence
  Primer VH1-FR1
ggcctcagtgaaggtctcctgcaag

SEQ ID NO: 2 - DNA, 25 bp, Artificial Sequence
  Primer VH2-FR1
gtctggtcctacgctggtgaaaccc

SEQ ID NO: 3 - DNA, 25 bp, Artificial Sequence
  Primer VH3-FR1
ctggggggtccctgagactctcctg

SEQ ID NO: 4 - DNA, 25 bp, Artificial Sequence
  Primer VH4-FR1
cttcggagaccctgtccctcacctg

SEQ ID NO: 5 - DNA, 25 bp, Artificial Sequence
  Primer VH5-FR1
cggggagtctctgaagatctcctgt

SEQ ID NO: 6 - DNA, 25 bp, Artificial Sequence
  Primer VH6-FR1
tcgcagaccctctcactcacctgtg

SEQ ID NO: 7 - DNA, 25 bp, Artificial Sequence
  Primer VH1-FR2
ctgggtgcgacaggcccctggacaa

SEQ ID NO: 8 - DNA, 25 bp, Artificial Sequence
  Primer VH2-FR2
tggatccgtcagcccccagggaagg

SEQ ID NO: 9 - DNA, 21 bp, Artificial Sequence
  Primer VH3-FR2
ggtccgccaggctccagggaa

SEQ ID NO: 10 - DNA, 25 bp, Artificial Sequence
  Primer VH4-FR2
tggatccgccagcccccagggaagg

SEQ ID NO: 11 - DNA, 25 bp, Artificial Sequence
  Primer VH5-FR2
gggtgcgccagatgcccgggaaagg

SEQ ID NO: 12 - DNA, 25 bp, Artificial Sequence
  Primer VH6-FR2
tggatcaggcagtccccatcgagag

SEQ ID NO: 13 - DNA, 25 bp, Artificial Sequence
  Primer VH7-FR2
ttgggtgcgacaggcccctggacaa

SEQ ID NO: 14 - DNA, 25 bp, Artificial Sequence
  Primer VH1-FR3
tggagctgagcagcctgagatctga

SEQ ID NO: 15 - DNA, 25 bp, Artificial Sequence
  Primer VH2-FR3
caatgaccaacatggaccctgtgga

SEQ ID NO: 16 - DNA, 25 bp, Artificial Sequence
  Primer VH3-FR3
tctgcaaatgaacagcctgagagcc

SEQ ID NO: 17 - DNA, 25 bp, Artificial Sequence
  Primer VH4-FR3
gagctctgtgaccgccgcggacacg

SEQ ID NO: 18 - DNA, 25 bp, Artificial Sequence
  Primer VH5-FR3
cagcaccgcctacctgcagtggagc

SEQ ID NO: 19 - DNA, 25 bp, Artificial Sequence
  Primer VH6-FR3
gttctccctgcagctgaactctgtg

SEQ ID NO: 20 - DNA, 24 bp, Artificial Sequence
  Primer VH7-FR3
cagcacggcatatctgcagatcag

SEQ ID NO: 21 - DNA, 18 bp, Artificial Sequence
  Primer DH1
ggcggaatgtgtgcaggc

SEQ ID NO: 22 - DNA, 21 bp, Artificial Sequence
  Primer DH2
gcactgggctcagagtcctct

SEQ ID NO: 23 - DNA, 20 bp, Artificial Sequence
  Primer DH3
gtggccctgggaatataaaa

SEQ ID NO: 24 - DNA, 19 bp, Artificial Sequence
  Primer DH4
agatccccaggacgcagca

SEQ ID NO: 25 - DNA, 20 bp, Artificial Sequence
  Primer DH5
cagggggacactgtgcatgt

SEQ ID NO: 26 - DNA, 19 bp, Artificial Sequence
  Primer DH6
tgaccccagcaagggaagg

SEQ ID NO: 27 - DNA, 18 bp, Artificial Sequence
  Primer DH7
cacaggccccctaccagc

SEQ ID NO: 28 - DNA, 22 bp, Artificial Sequence
  Primer JH57
cttacctgaggagacggtgacc

SEQ ID NO: 29 - DNA, 25 bp, Artificial Sequence
  Primer VK1f/6
tcaaggttcagcggcagtggatctg

SEQ ID NO: 30 - DNA, 26 bp, Artificial Sequence
  Primer VK2f
ggcctccatctcctgcaggtctagtc

SEQ ID NO: 31 - DNA, 27 bp, Artificial Sequence
  Primer VK3f
cccaggctcctcatctatgatgcatcc

SEQ ID NO: 32 - DNA, 27 bp, Artificial Sequence
  Primer VK4
caactgcaagtccagccagagtgtttt

SEQ ID NO: 33 - DNA, 26 bp, Artificial Sequence
  Primer VK5
cctgcaaagccagccaagacattgat

SEQ ID NO: 34 - DNA, 27 bp, Artificial Sequence
  Primer VK6
gaccgatttcaccctcacaattaatcc

SEQ ID NO: 35 - DNA, 27 bp, Artificial Sequence
  Primer JK1-4
cttacgtttgatctccaccttggtccc

SEQ ID NO: 36 - DNA, 27 bp, Artificial Sequence
  Primer JK5
cttacgtttaatctccagtcgtgtccc

SEQ ID NO: 37 - DNA, 27 bp, Artificial Sequence
  Primer Kde
cctcagaggtcagagcaggttgtccta

SEQ ID NO: 38 - DNA, 22 bp, Artificial Sequence
  Primer INTR
cgtggcaccgcgagctgtagac

SEQ ID NO: 39 - DNA, 27 bp, Artificial Sequence
  Forward primer for TP53
aaggtgataaaagtgaatctgaggcat

SEQ ID NO: 40 - DNA, 22 bp, Artificial Sequence
  Reverse primer for TP53
aatgggacaggtaggacctgat

SEQ ID NO: 41 - DNA, 22 bp, Artificial Sequence
  Forward primer for TP53
ctgctcaccatcgctatctgag

SEQ ID NO: 42 - DNA, 26 bp, Artificial Sequence
  Reverse primer for TP53
ctttcaactctgtctccttcctcttc

SEQ ID NO: 43 - DNA, 22 bp, Artificial Sequence
  Forward primer for TP53
tgtgatgagaggtggatgggta

SEQ ID NO: 44 - DNA, 22 bp, Artificial Sequence
  Reverse primer for TP53
cctcatcttgggcctgtgttat

SEQ ID NO: 45 - DNA, 22 bp, Artificial Sequence
  Forward primer for TP53
tcatagggcaccaccacactat

SEQ ID NO: 46 - DNA, 22 bp, Artificial Sequence
  Reverse primer for TP53
tacaagcagtcacagcacatga

SEQ ID NO: 47 - DNA, 22 bp, Artificial Sequence
  Forward primer for TP53
cttgcttacctcgcttagtgct

SEQ ID NO: 48 - DNA, 27 bp, Artificial Sequence
  Reverse primer for TP53
gcttctcttttcctatcctgagtagtg

SEQ ID NO: 49 - DNA, 20 bp, Artificial Sequence
  Forward primer for TP53
ggctcctgacctggagtctt

SEQ ID NO: 50 - DNA, 19 bp, Artificial Sequence
  Reverse primer for TP53
aaggcgcactggcctcatc

SEQ ID NO: 51 - DNA, 22 bp, Artificial Sequence
  Forward primer for TP53
ggccagacctaagagcaatcag

SEQ ID NO: 52 - DNA, 22 bp, Artificial Sequence
  Reverse primer for TP53
catggccatctacaagcagtca

SEQ ID NO: 53 - DNA, 19 bp, Artificial Sequence
  Forward primer for TP53
acaacctccgtcatgtgct

SEQ ID NO: 54 - DNA, 26 bp, Artificial Sequence
  Reverse primer for TP53
gtctccttcctcttcctacagtactc

SEQ ID NO: 55 - DNA, 29 bp, Artificial Sequence
  Forward primer for NRAS
gctcctagtacctgtagaggttaatatcc

SEQ ID NO: 56 - DNA, 28 bp, Artificial Sequence
  Reverse primer for NRAS
gttatagatggtgaaacctgtttgttgg

SEQ ID NO: 57 - DNA, 22 bp, Artificial Sequence
  Forward primer for NRAS
cgacaagtgagagacaggatca

SEQ ID NO: 58 - DNA, 24 bp, Artificial Sequence
  Reverse primer for NRAS
tcttgctggtgtgaaatgactgag

SEQ ID NO: 59 - DNA, 23 bp, Artificial Sequence
  Forward primer for KRAS
caaagaatggtcctgcaccagta

SEQ ID NO: 60 - DNA, 27 bp, Artificial Sequence
  Reverse primer for KRAS
aaggcctgctgaaaatgactgaatata

SEQ ID NO: 61 - DNA, 23 bp, Artificial Sequence
  Forward primer for KRAS
gctgtatcgtcaaggcactcttg

SEQ ID NO: 62 - DNA, 30 bp, Artificial Sequence
  Reverse primer for KRAS
aggtactggtggagtatttgatagtgtatt

SEQ ID NO: 63 - DNA, 33 bp, Artificial Sequence
  Forward primer for KRAS
tgtcagcttattatattcaatttaaacccacct

SEQ ID NO: 64 - DNA, 24 bp, Artificial Sequence
  Reverse primer for KRAS
tcttggatattctcgacacagcag

SEQ ID NO: 65 - DNA, 28 bp, Artificial Sequence
  Forward primer for BRAF
ccttcaatgactttctagtaactcagca

SEQ ID NO: 66 - DNA, 30 bp, Artificial Sequence
  Reverse primer for BRAF
cttacctaaactcttcataatgcttgctct

SEQ ID NO: 67 - DNA, 25 bp, Artificial Sequence
  Forward primer for FLT3
ccctgacaacatagttggaatcact

SEQ ID NO: 68 - DNA, 30 bp, Artificial Sequence
  Reverse primer for FLT3
cactccaggataatacacatcacagtaaat

SEQ ID NO: 69 - DNA, 25 bp, Artificial Sequence
  Forward primer for SF3B1
caagatggcacagcccataagaata

SEQ ID NO: 70 - DNA, 22 bp, Artificial Sequence
  Reverse primer for SF3B1
agcttttgctgttgtagcctct

SEQ ID NO: 71 - DNA, 22 bp, Artificial Sequence
  Forward primer for SF3B1
caagatggcacagcccataaga

SEQ ID NO: 72 - DNA, 29 bp, Artificial Sequence
  Reverse primer for SF3B1
actcatgactgtcctttctttgtttacat

SEQ ID NO: 73 - DNA, 26 bp, Artificial Sequence
  Forward primer for SF3B1
aggtaattggtggatttacctttcct

SEQ ID NO: 74 - DNA, 27 bp, Artificial Sequence
  Reverse primer for SF3B1
ggcatagttaaaacctgtgtttggttt

SEQ ID NO: 75 - DNA, 25 bp, Artificial Sequence
  Forward primer for SF3B1
tcatttcctcatcaggagactggaa

SEQ ID NO: 76 - DNA, 28 bp, Artificial Sequence
  Reverse primer for SF3B1
tgtgttaaagcctttatggaagggtatc

SEQ ID NO: 77 - DNA, 22 bp, Artificial Sequence
  Forward primer for SF3B1
gttggcggatacccttccataa

SEQ ID NO: 78 - DNA, 28 bp, Artificial Sequence
  Reverse primer for SF3B1
ggcatagttaaaacctgtgtttggtttt

SEQ ID NO: 79 - DNA, 24 bp, Artificial Sequence
  Forward primer for EZH2
agttccaattctcacgtcaaaggt

SEQ ID NO: 80 - DNA, 25 bp, Artificial Sequence
  Reverse primer for EZH2
aattattcactgggctgtgcttact

SEQ ID NO: 81 - DNA, 22 bp, Artificial Sequence
  Forward primer for EZH2
agtgccttacctctccacagta

SEQ ID NO: 82 - DNA, 25 bp, Artificial Sequence
  Reverse primer for EZH2
ccagtccattttcaccctccttttt

SEQ ID NO: 83 - DNA, 19 bp, Artificial Sequence
  Forward primer for CREBBP
tcgccagagacaagcactg

SEQ ID NO: 84 - DNA, 18 bp, Artificial Sequence
  Reverse primer for CREBBP
gtgcagctccaccagcat

SEQ ID NO: 85 - DNA, 18 bp, Artificial Sequence
  Forward primer for BCL2
gcacctgacgcccttcac

SEQ ID NO: 86 - DNA, 20 bp, Artificial Sequence
  Reverse primer for BCL2
aagaaggccacaatcctccc

SEQ ID NO: 87 - DNA, 17 bp, Artificial Sequence
  Forward primer for MYD88
ttggcttgcaggtgccc

SEQ ID NO: 88 - DNA, 20 bp, Artificial Sequence
  Reverse primer for MYD88
ggttggtgtagtcgcagaca

SEQ ID NO: 89 - DNA, 20 bp, Artificial Sequence
  Forward primer for BTK
tctttcccatgagaagctgg

SEQ ID NO: 90 - DNA, 20 bp, Artificial Sequence
  Reverse primer for BTK
catccttgcacatctctagc

SEQ ID NO: 91 - DNA, 20 bp, Artificial Sequence
  Forward primer for NOTCH1
gaactgaggcctgagagctt

SEQ ID NO: 92 - DNA, 20 bp, Artificial Sequence
  Reverse primer for NOTCH1
cagacctgtgaggtcgacat

SEQ ID NO: 93 - DNA, 18 bp, Artificial Sequence
  Forward primer for NOTCH1
gtcccgcagacatcctga

SEQ ID NO: 94 - DNA, 20 bp, Artificial Sequence
  Reverse primer for NOTCH1
ggtggccgatttgggagatc

SEQ ID NO: 95 - DNA, 19 bp, Artificial Sequence
  Forward primer for NOTCH1
ccgaaggcttgggaaagga

SEQ ID NO: 96 - DNA, 19 bp, Artificial Sequence
  Reverse primer for NOTCH1
cctcgcctgtggacaacac

SEQ ID NO: 97 - DNA, 22 bp, Artificial Sequence
  Forward primer for XPO1
ctccaacctgaacctgaacgaa

SEQ ID NO: 98 - DNA, 29 bp, Artificial Sequence
  Reverse primer for XPO1
ctcactggaaatttctgaagactgtagtt

SEQ ID NO: 99 - DNA, 28 bp, Artificial Sequence
  Forward primer for BIRC3
ctttagtagaagcctggtaaaacagaca

SEQ ID NO: 100 - DNA, 30 bp, Artificial Sequence
  Reverse primer for BIRC3
aaaaacctgactggattgagtatattttca

SEQ ID NO: 101 - DNA, 30 bp, Artificial Sequence
  Forward primer for BIRC3
ttcttagtttttcactgaagaagcaaactg

SEQ ID NO: 102 - DNA, 29 bp, Artificial Sequence
  Reverse primer for BIRC3
tggttcttcttcatgaaagaaatgtacga

SEQ ID NO: 103 - DNA, 22 bp, Artificial Sequence
  Forward primer for EGR2
tctgtctcaggtggatcttggt

SEQ ID NO: 104 - DNA, 21 bp, Artificial Sequence
  Reverse primer for EGR2
tgaccacctcaccacccatat

SEQ ID NO: 105 - DNA, 24 bp, Artificial Sequence
  Forward primer for FBXW7
tttttggactgtactggatcagca

SEQ ID NO: 106 - DNA, 24 bp, Artificial Sequence
  Reverse primer for FBXW7
catgttttgatgggtcatgttgca

SEQ ID NO: 107 - DNA, 24 bp, Artificial Sequence
  Forward primer for FBXW7
tagaggaagaagtcccaaccatga

SEQ ID NO: 108 - DNA, 30 bp, Artificial Sequence
  Reverse primer for FBXW7
tcacttttcctttctacccaaaagtaatca

SEQ ID NO: 109 - DNA, 22 bp, Artificial Sequence
  Forward primer for FBXW7
caactgtccttgctgggaatca

SEQ ID NO: 110 - DNA, 22 bp, Artificial Sequence
  Reverse primer for FBXW7
caagaagtagcaagctggcttt

SEQ ID NO: 111 - DNA, 21 bp, Artificial Sequence
  Forward primer for NFKBIE
gggacttgaaggatcttcacg

SEQ ID NO: 112 - DNA, 21 bp, Artificial Sequence
  Reverse primer for NFKBIE
ggctgattccacctatggctc

SEQ ID NO: 113 - DNA, 32 bp, Artificial Sequence
  Forward primer for IDH1
aagaataaaacacatacaagttggaaatttct

SEQ ID NO: 114 - DNA, 28 bp, Artificial Sequence
  Reverse primer for IDH1
gagaagccattatctgcaaaaatatccc

SEQ ID NO: 115 - DNA, 20 bp, Artificial Sequence
  Forward primer for IDH2
ggactaggcgtgggatgttt

SEQ ID NO: 116 - DNA, 26 bp, Artificial Sequence
  Reverse primer for IDH2
gggttcaaattctggttgaaagatgg

SEQ ID NO: 117 - DNA, 31 bp, Artificial Sequence
  Forward primer for U2AF1
attaactgtctttgaaaagaacatgaagttt

SEQ ID NO: 118 - DNA, 28 bp, Artificial Sequence
  Reverse primer for U2AF1
tttcccttacagagtcaactgttcattt

SEQ ID NO: 119 - DNA, 24 bp, Artificial Sequence
  Forward primer for RUNX1
aatctgagacatggtccctgagta

SEQ ID NO: 120 - DNA, 23 bp, Artificial Sequence
  Reverse primer for RUNX1
ccatcactgtcttcacaaaccca

SEQ ID NO: 121 - DNA, 23 bp, Artificial Sequence
  Forward primer for RUNX1
agaccgagtttctagggattcca

SEQ ID NO: 122 - DNA, 23 bp, Artificial Sequence
  Reverse primer for RUNX1
ctaccgcagccatgaagaaccag

SEQ ID NO: 123 - DNA, 33 bp, Artificial Sequence
  Forward primer for KIT
aatgaaagttaatatggagaagttaattgctgc

SEQ ID NO: 124 - DNA, 29 bp, Artificial Sequence
  Reverse primer for KIT
gtgatgccagctattatatttctcctgta

SEQ ID NO: 125 - DNA, 32 bp, Artificial Sequence
  Forward primer for KIT
tgaatttaaatggttttcttttctcctccaac

SEQ ID NO: 126 - DNA, 33 bp, Artificial Sequence
  Reverse primer for KIT
cacgtttcctttaaccacataattagaatcatt

SEQ ID NO: 127 - DNA, 26 bp, Artificial Sequence
  Forward primer for KIT
attttggtctagccagagacatcaag

SEQ ID NO: 128 - DNA, 30 bp, Artificial Sequence
  Reverse primer for KIT
tgtgtgatatccctagacaggatttacatt

SEQ ID NO: 129 - DNA, 22 bp, Artificial Sequence
  Forward primer for KIT
tggatggcacctgaaagcattt

SEQ ID NO: 130 - DNA, 29 bp, Artificial Sequence
  Reverse primer for KIT
gaaacttcaagaagatgctctgagtctaa